European Patent Application EP 4 454 658 A1, published October 30, 2024. Title: Hepatic targeting drug and use thereof. Applicant: HANMI PHARM. CO., LTD. The sequence listing filed with the application follows.

SEQUENCE LISTING (140 sequences)

SEQ ID NO: 1 - protein, 30 aa, synthetic construct
  REGION 1..30: note = Trigonal agonist
  SITE 2: note = X is aminoisobutyric acid (Aib)
HXQGTFTSDVSSYLDGQAAKEFIAWLVKGC

SEQ ID NO: 2 - protein, 30 aa, synthetic construct
  REGION 1..30: note = Trigonal agonist
  SITE 2: note = X is aminoisobutyric acid (Aib)
HXQGTFTSDVSSYLDGQAQKEFIAWLVKGC

SEQ ID NO: 3 - protein, 41 aa, synthetic construct
  REGION 1..41: note = Trigonal agonist
  SITE 2: note = X is aminoisobutyric acid (Aib)
HXQGTFTSDVSSYLLGQAAKQFIAWLVKGGGPSSGAPPPSC

SEQ ID NO: 4 - protein, 30 aa, synthetic construct
  REGION 1..30: note = Trigonal agonist
  SITE 2: note = X is aminoisobutyric acid (Aib)
HXQGTFTSDVSSYLLGQQQKEFIAWLVKGC

SEQ ID NO: 5 - protein, 41 aa, synthetic construct
  REGION 1..41: note = Trigonal agonist
  SITE 2: note = X is aminoisobutyric acid (Aib)
HXQGTFTSDVSSYLLGQQQKEFIAWLVKGGGPSSGAPPPSC

SEQ ID NO: 6 - protein, 30 aa, synthetic construct
  REGION 1..30: note = Trigonal agonist
  SITE 2: note = X is aminoisobutyric acid (Aib)
HXQGTFTSDVSSYLDGQAAKEFVAWLLKGC

SEQ ID NO: 7 - protein, 30 aa, synthetic construct
  REGION 1..30: note = Trigonal agonist
  SITE 2: note = X is aminoisobutyric acid (Aib)
HXQGTFTSDVSKYLDGQAAKEFVAWLLKGC

SEQ ID NO: 8 - protein, 30 aa, synthetic construct
  REGION 1..30: note = Trigonal agonist
  SITE 2: note = X is aminoisobutyric acid (Aib)
HXQGTFTSDVSKYLDGQAAQEFVAWLLKGC

SEQ ID NO: 9 - protein, 30 aa, synthetic construct
  REGION 1..30: note = Trigonal agonist
  SITE 2: note = X is aminoisobutyric acid (Aib)
HXQGTFTSDVSKYLDGQAAQEFVAWLLAGC

SEQ ID NO: 10 - protein, 41 aa, synthetic construct
  REGION 1..41: note = Trigonal agonist
  SITE 2: note = X is aminoisobutyric acid (Aib)
HXQGTFTSDVSKYLDGQAAQEFVAWLLAGGGPSSGAPPPSC

SEQ ID NO: 11 - protein, 41 aa, synthetic construct
  REGION 1..41: note = Trigonal agonist
  SITE 1: note = X is 4-imidazoacetyl (CA)
XGEGTFTSDLSKYLDSRRQQLFVQWLKAGGPSSGAPPPSHG

SEQ ID NO: 12 - protein, 41 aa, synthetic construct
  REGION 1..41: note = Trigonal agonist
  SITE 1: note = X is 4-imidazoacetyl (CA)
XGEGTFISDLSKYMDEQAVQLFVEWLMAGGPSSGAPPPSHG

SEQ ID NO: 13 - protein, 41 aa, synthetic construct
  REGION 1..41: note = Trigonal agonist
  SITE 1: note = X is 4-imidazoacetyl (CA)
XGEGTFISDYSIQLDEIAVQDFVEWLLAQKPSSGAPPPSHG

SEQ ID NO: 14 - protein, 41 aa, synthetic construct
  REGION 1..41: note = Trigonal agonist
  SITE 1: note = X is 4-imidazoacetyl (CA)
XGQGTFTSDYSIQLDEIAVRDFVEWLKNGGPSSGAPPPSHG

SEQ ID NO: 15 - protein, 41 aa, synthetic construct
  REGION 1..41: note = Trigonal agonist
  SITE 1: note = X is 4-imidazoacetyl (CA)
XGQGTFTSDLSKQMDEEAVRLFIEWLKNGGPSSGAPPPSHG

SEQ ID NO: 16 - protein, 41 aa, synthetic construct
  REGION 1..41: note = Trigonal agonist
  SITE 1: note = X is 4-imidazoacetyl (CA)
XGQGTFTSDLSKQMDSEAQQLFIEWLKNGGPSSGAPPPSHG

SEQ ID NO: 17 - protein, 41 aa, synthetic construct
  REGION 1..41: note = Trigonal agonist
  SITE 1: note = X is 4-imidazoacetyl (CA)
XGQGTFTSDLSKQMDEERAREFIEWLLAQKPSSGAPPPSHG

SEQ ID NO: 18 - protein, 41 aa, synthetic construct
  REGION 1..41: note = Trigonal agonist
  SITE 1: note = X is 4-imidazoacetyl (CA)
XGQGTFTSDLSKQMDSERAREFIEWLKNTGPSSGAPPPSHG

SEQ ID NO: 19 - protein, 41 aa, synthetic construct
  REGION 1..41: note = Trigonal agonist
  SITE 1: note = X is 4-imidazoacetyl (CA)
XGQGTFTSDLSIQYDSEHQRDFIEWLKDTGPSSGAPPPSHG

SEQ ID NO: 20 - protein, 41 aa, synthetic construct
  REGION 1..41: note = Trigonal agonist
  SITE 1: note = X is 4-imidazoacetyl (CA)
XGQGTFTSDLSIQYEEEAQQDFVEWLKDTGPSSGAPPPSHG

SEQ ID NO: 21 - protein, 39 aa, synthetic construct
  REGION 1..39: note = Trigonal agonist
  SITE 2: note = X is aminoisobutyric acid (Aib)
  SITE 16..20: note = amino acids at positions 16 and 20 together form a ring
YXQGTFTSDYSKYLDECRAKEFVQWLLDHHPSSGQPPPS

SEQ ID NO: 22 - protein, 39 aa, synthetic construct
  REGION 1..39: note = Trigonal agonist
  SITE 2: note = X is aminoisobutyric acid (Aib)
  SITE 16..20: note = amino acids at positions 16 and 20 together form a ring
YXQGTFTSDYSKCLDEKRAKEFVQWLLDHHPSSGQPPPS

SEQ ID NO: 23 - protein, 41 aa, synthetic construct
  REGION 1..41: note = Trigonal agonist
  SITE 2: note = X is aminoisobutyric acid (Aib)
  REGION 16..20: note = amino acids at positions 16 and 20 together form a ring
YXQGTFTSDYSKYLDECRAKEFVQWLLAQKGKKNDWKHNIT

SEQ ID NO: 24 - protein, 39 aa, synthetic construct
  REGION 1..39: note = Trigonal agonist
  SITE 2: note = X is aminoisobutyric acid (Aib)
  SITE 16..20: note = amino acids at positions 16 and 20 together form a ring
YXQGTFTSDYSKYLDECRAKEFVQWLKNGGPSSGAPPPS

SEQ ID NO: 25 - protein, 39 aa, synthetic construct
  REGION 1..39: note = Trigonal agonist
  SITE 2: note = X is aminoisobutyric acid (Aib)
HXQGTFTSDCSKYLDERAAQDFVQWLLDGGPSSGAPPPS

SEQ ID NO: 26 - protein, 39 aa, synthetic construct
  REGION 1..39: note = Trigonal agonist
  SITE 2: note = X is aminoisobutyric acid (Aib)
HXQGTFTSDCSKYLDSRAAQDFVQWLLDGGPSSGAPPPS

SEQ ID NO: 27 - protein, 40 aa, synthetic construct
  REGION 1..40: note = Trigonal agonist
  SITE 2: note = X is aminoisobutyric acid (Aib)
HXQGTFTSDYSKYLDERACQDFVQWLLDQGGPSSGAPPPS

SEQ ID NO: 28 - protein, 41 aa, synthetic construct
  REGION 1..41: note = Trigonal agonist
  SITE 2: note = X is aminoisobutyric acid (Aib)
HXQGTFTSDYSKYLDEKRAQEFVCWLLAQKGKKNDWKHNIT

SEQ ID NO: 29 - protein, 30 aa, synthetic construct
  REGION 1..30: note = Trigonal agonist
  SITE 2: note = X is aminoisobutyric acid (Aib)
  SITE 16..20: note = amino acids at positions 16 and 20 together form a ring
HXQGTFTSDYSKYLDEKAAKEFVQWLLNTC

SEQ ID NO: 30 - protein, 30 aa, synthetic construct
  REGION 1..30: note = Trigonal agonist
  SITE 2: note = X is aminoisobutyric acid (Aib)
  REGION 16..20: note = amino acids at positions 16 and 20 together form a ring
HXQGTFTSDYSKYLDEKAQKEFVQWLLDTC

SEQ ID NO: 31 - protein, 29 aa, synthetic construct
  REGION 1..29: note = Trigonal agonist
  SITE 2: note = X is aminoisobutyric acid (Aib)
  SITE 16..20: note = amino acids at positions 16 and 20 together form a ring
HXQGTFTSDYSKYLDEKACKEFVQWLLAQ

SEQ ID NO: 32 - protein, 39 aa, synthetic construct
  REGION 1..39: note = Trigonal agonist
  SITE 2: note = X is aminoisobutyric acid (Aib)
  SITE 16..20: note = amino acids at positions 16 and 20 together form a ring
HXQGTFTSDYSKYLDEKACKDFVQWLLDGGPSSGAPPPS

SEQ ID NO: 33 - protein, 31 aa, synthetic construct
  REGION 1..31: note = Trigonal agonist
  SITE 2: note = X is aminoisobutyric acid (Aib)
  SITE 16..20: note = amino acids at positions 16 and 20 together form a ring
HXQGTFTSDYSIAMDEIHQKDFVNWLLAQKC

SEQ ID NO: 34 - protein, 31 aa, synthetic construct
  REGION 1..31: note = Trigonal agonist
  SITE 2: note = X is aminoisobutyric acid (Aib)
  SITE 16..20: note = amino acids at positions 16 and 20 together form a ring
HXQGTFTSDYSKYLDEKRQKEFVNWLLAQKC

SEQ ID NO: 35 - protein, 31 aa, synthetic construct
  REGION 1..31: note = Trigonal agonist
  SITE 2: note = X is aminoisobutyric acid (Aib)
  REGION 16..20: note = amino acids at positions 16 and 20 together form a ring
HXQGTFTSDYSIAMDEIHQKDFVNWLLNTKC

SEQ ID NO: 36 - protein, 40 aa, synthetic construct
  REGION 1..40: note = Trigonal agonist
  SITE 2: note = X is aminoisobutyric acid (Aib)
  SITE 16..20: note = amino acids at positions 16 and 20 together form a ring
HXQGTFTSDYSKYLCEKRQKEFVQWLLNGGPSSGAPPPSG

SEQ ID NO: 37 - protein, 40 aa, synthetic construct
  REGION 1..40: note = Trigonal agonist
  SITE 2: note = X is aminoisobutyric acid (Aib)
  SITE 16..20: note = amino acids at positions 16 and 20 together form a ring
HXQGTFTSDYSKYLDECRQKEFVQWLLNGGPSSGAPPPSG

SEQ ID NO: 38 - protein, 40 aa, synthetic construct
  REGION 1..40: note = Trigonal agonist
  SITE 1: note = X is 4-imidazoacetyl (CA)
  SITE 2: note = X is aminoisobutyric acid (Aib)
XXQGTFTSDKSSYLDERAAQDFVQWLLDGGPSSGAPPPSS

SEQ ID NO: 39 - protein, 40 aa, synthetic construct
  REGION 1..40: note = Trigonal agonist
  SITE 2: note = X is aminoisobutyric acid (Aib)
HXQGTFTSDYSKYLDGQHAQCFVAWLLAGGGPSSGAPPPS

SEQ ID NO: 40 - protein, 39 aa, synthetic construct
  REGION 1..39: note = Trigonal agonist
  SITE 2: note = X is aminoisobutyric acid (Aib)
HXQGTFTSDKSKYLDERACQDFVQWLLDGGPSSGAPPPS

SEQ ID NO: 41 - protein, 39 aa, synthetic construct
  REGION 1..39: note = Trigonal agonist
  SITE 2: note = X is aminoisobutyric acid (Aib)
HXQGTFTSDKSKYLDECAAQDFVQWLLDGGPSSGAPPPS

SEQ ID NO: 42 - protein, 40 aa, synthetic construct
  REGION 1..40: note = Trigonal agonist
  SITE 2: note = X is aminoisobutyric acid (Aib)
  SITE 16..20: note = amino acids at positions 16 and 20 together form a ring
YXQGTFTSDYSKYLDEKRAKEFVQWLLDHHPSSGQPPPSC

SEQ ID NO: 43 - protein, 39 aa, synthetic construct
  REGION 1..39: note = Trigonal agonist
  SITE 2: note = X is aminoisobutyric acid (Aib)
  SITE 16..20: note = amino acids at positions 16 and 20 together form a ring
YXQGTFTSDYSKYLDEKRAKEFVQWLLDHHCSSGQPPPS

SEQ ID NO: 44 - protein, 39 aa, synthetic construct
  REGION 1..39: note = Trigonal agonist
HGQGTFTSDCSKQLDGQAAQEFVAWLLAGGPSSGAPPPS

SEQ ID NO: 45 - protein, 39 aa, synthetic construct
  REGION 1..39: note = Trigonal agonist
HGQGTFTSDCSKYMDGQAAQDFVAWLLAGGPSSGAPPPS

SEQ ID NO: 46 - protein, 39 aa, synthetic construct
  REGION 1..39: note = Trigonal agonist
HGQGTFTSDCSKYLDEQHAQEFVAWLLAGGPSSGAPPPS

SEQ ID NO: 47 - protein, 39 aa, synthetic construct
  REGION 1..39: note = Trigonal agonist
HGQGTFTSDCSKYLDGQRAQEFVAWLLAGGPSSGAPPPS

SEQ ID NO: 48 - protein, 39 aa, synthetic construct
  REGION 1..39: note = Trigonal agonist
HGQGTFTSDCSKYLDGQRAQDFVNWLLAGGPSSGAPPPS

SEQ ID NO: 49 - protein, 30 aa, synthetic construct
  REGION 1..30: note = Trigonal agonist
  SITE 1: note = X is 4-imidazoacetyl (CA)
  SITE 2: note = X is aminoisobutyric acid (Aib)
  SITE 16..20: note = amino acids at positions 16 and 20 together form a ring
XXQGTFTSDYSICMDEIHQKDFVNWLLNTK

SEQ ID NO: 50 - protein, 40 aa, synthetic construct
  REGION 1..40: note = Trigonal agonist
  SITE 2: note = X is aminoisobutyric acid (Aib)
  REGION 16..20: note = amino acids at positions 16 and 20 together form a ring
HXQGTFTSDYSKYLDEKRAKEFVQWLLDHHPSSGQPPPSC

SEQ ID NO: 51 - protein, 30 aa, synthetic construct
  REGION 1..30: note = Trigonal agonist
  SITE 2: note = X is aminoisobutyric acid (Aib)
  SITE 16..20: note = amino acids at positions 16 and 20 together form a ring
HXQGTFTSDYSKYLDEKRQKEFVQWLLNTC

SEQ ID NO: 52 - protein, 30 aa, synthetic construct
  REGION 1..30: note = Trigonal agonist
  SITE 2: note = X is aminoisobutyric acid (Aib)
  SITE 16..20: note = amino acids at positions 16 and 20 together form a ring
HXQGTFTSDYSKYLDEKRQKEFVQWLLDTC

SEQ ID NO: 53 - protein, 30 aa, synthetic construct
  REGION 1..30: note = Trigonal agonist
  SITE 2: note = X is aminoisobutyric acid (Aib)
  SITE 16..20: note = amino acids at positions 16 and 20 together form a ring
HXEGTFTSDYSIAMDEIHQKDFVNWLLAQC

SEQ ID NO: 54 - protein, 30 aa, synthetic construct
  REGION 1..30: note = Trigonal agonist
  SITE 2: note = X is aminoisobutyric acid (Aib)
  SITE 16..20: note = amino acids at positions 16 and 20 together form a ring
HXEGTFTSDYSIAMDEIHQKDFVDWLLAEC

SEQ ID NO: 55 - protein, 30 aa, synthetic construct
  REGION 1..30: note = Trigonal agonist
  SITE 2: note = X is aminoisobutyric acid (Aib)
  SITE 16..20: note = amino acids at positions 16 and 20 together form a ring
HXQGTFTSDYSIAMDEIHQKDFVNWLLAQC

SEQ ID NO: 56 - protein, 30 aa, synthetic construct
  REGION 1..30: note = Trigonal agonist
  SITE 2: note = X is aminoisobutyric acid (Aib)
  SITE 16..20: note = amino acids at positions 16 and 20 together form a ring
HXQGTFTSDYSKYLDEKRQKEFVNWLLAQC

SEQ ID NO: 57 - protein, 30 aa, synthetic construct
  REGION 1..30: note = Trigonal agonist
  SITE 2: note = X is aminoisobutyric acid (Aib)
  SITE 16..20: note = amino acids at positions 16 and 20 together form a ring
HXQGTFTSDYSIAMDEIHQKDFVNWLLNTC

SEQ ID NO: 58 - protein, 31 aa, synthetic construct
  REGION 1..31: note = Trigonal agonist
  SITE 2: note = X is aminoisobutyric acid (Aib)
  SITE 16..20: note = amino acids at positions 16 and 20 together form a ring
HXQGTFTSDYSKYLDEKRQKEFVQWLLNTKC

SEQ ID NO: 59 - protein, 30 aa, synthetic construct
  REGION 1..30: note = Trigonal agonist
  SITE 1: note = X is 4-imidazoacetyl (CA)
  SITE 2: note = X is aminoisobutyric acid (Aib)
  SITE 16..20: note = amino acids at positions 16 and 20 together form a ring
XXQGTFTSDYSICMDEKHQKDFVNWLLNTK

SEQ ID NO: 60 - protein, 30 aa, synthetic construct
  REGION 1..30: note = Trigonal agonist
  SITE 1: note = X is 4-imidazoacetyl (CA)
  SITE 2: note = X is aminoisobutyric acid (Aib)
  SITE 16..20: note = amino acids at positions 16 and 20 together form a ring
XXQGTFTSDYSIAMDEKHCKDFVNWLLNTK

SEQ ID NO: 61 - protein, 30 aa, synthetic construct
  REGION 1..30: note = Trigonal agonist
  SITE 1: note = X is 4-imidazoacetyl (CA)
  SITE 2: note = X is aminoisobutyric acid (Aib)
  SITE 16..20: note = amino acids at positions 16 and 20 together form a ring
XXQGTFTSDYSIAMDEIACKDFVNWLLNTK

SEQ ID NO: 62 - protein, 39 aa, synthetic construct
  REGION 1..39: note = Trigonal agonist
  SITE 1: note = X is 4-imidazoacetyl (CA)
  SITE 2: note = X is aminoisobutyric acid (Aib)
XXQGTFTSDKSKYLDERAAQDFVQWLLDGGPSSGAPPPS

SEQ ID NO: 63 - protein, 39 aa, synthetic construct
  REGION 1..39: note = Trigonal agonist
  SITE 1: note = X is 4-imidazoacetyl (CA)
  SITE 2: note = X is aminoisobutyric acid (Aib)
XXQGTFTSDCSKYLDERAAQDFVQWLLDGGPSSGAPPPS

SEQ ID NO: 64 - protein, 39 aa, synthetic construct
  REGION 1..39: note = Trigonal agonist
  SITE 2: note = X is aminoisobutyric acid (Aib)
  SITE 16..20: note = amino acids at positions 16 and 20 together form a ring
YXQGTFTSDYSKYLDECAAKEFVQWLLDHHPSSGQPPPS

SEQ ID NO: 65 - protein, 39 aa, synthetic construct
  REGION 1..39: note = Trigonal agonist
  SITE 2: note = X is aminoisobutyric acid (Aib)
  SITE 16..20: note = amino acids at positions 16 and 20 together form a ring
HXQGTFTSDYSKCLDEKRAKEFVQWLLDHHPSSGQPPPS

SEQ ID NO: 66 - protein, 39 aa, synthetic construct
  REGION 1..39: note = Trigonal agonist
  SITE 2: note = X is aminoisobutyric acid (Aib)
  SITE 16..20: note = amino acids at positions 16 and 20 together form a ring
YXQGTFTSDYSKYLDECRAKDFVQWLLDHHPSSGQPPPS

SEQ ID NO: 67 - protein, 39 aa, synthetic construct
  REGION 1..39: note = Trigonal agonist
  SITE 2: note = X is aminoisobutyric acid (Aib)
  SITE 16..20: note = amino acids at positions 16 and 20 together form a ring
YXQGTFTSDYSKYLDECAAKDFVQWLLDHHPSSGQPPPS

SEQ ID NO: 68 - protein, 39 aa, synthetic construct
  REGION 1..39: note = Trigonal agonist
  SITE 2: note = X is aminoisobutyric acid (Aib)
  SITE 16..20: note = amino acids at positions 16 and 20 together form a ring
YXQGTFTSDYSKCLDEKAAKEFVQWLLDHHPSSGQPPPS

SEQ ID NO: 69 - protein, 39 aa, synthetic construct
  REGION 1..39: note = Trigonal agonist
  SITE 2: note = X is aminoisobutyric acid (Aib)
  SITE 16..20: note = amino acids at positions 16 and 20 together form a ring
YXQGTFTSDYSKCLDERAAKEFVQWLLDHHPSSGQPPPS

SEQ ID NO: 70 - protein, 39 aa, synthetic construct
  REGION 1..39: note = Trigonal agonist
  SITE 2: note = X is aminoisobutyric acid (Aib)
  SITE 16..20: note = amino acids at positions 16 and 20 together form a ring
YXQGTFTSDYSKCLDEKRAKDFVQWLLDHHPSSGQPPPS

SEQ ID NO: 71 - protein, 39 aa, synthetic construct
  REGION 1..39: note = Trigonal agonist
  SITE 2: note = X is aminoisobutyric acid (Aib)
  SITE 16..20: note = amino acids at positions 16 and 20 together form a ring
YXQGTFTSDYSKYLDERACKDFVQWLLDHHPSSGQPPPS

SEQ ID NO: 72 - protein, 39 aa, synthetic construct
  REGION 1..39: note = Trigonal agonist
  SITE 2: note = X is aminoisobutyric acid (Aib)
  SITE 16..20: note = amino acids at positions 16 and 20 together form a ring
YXQGTFTSDCSKYLDERAAKDFVQWLLDHHPSSGQPPPS

SEQ ID NO: 73 - protein, 39 aa, synthetic construct
  REGION 1..39: note = Trigonal agonist
  SITE 1: note = X is 4-imidazoacetyl (CA)
  SITE 2: note = X is aminoisobutyric acid (Aib)
  SITE 16..20: note = amino acids at positions 16 and 20 together form a ring
XXQGTFTSDYSKYLDECRAKEFVQWLLDHHPSSGQPPPS

SEQ ID NO: 74 - protein, 39 aa, synthetic construct
  REGION 1..39: note = Trigonal agonist
  SITE 1: note = X is 4-imidazoacetyl (CA)
  SITE 2: note = X is aminoisobutyric acid (Aib)
  SITE 16..20: note = amino acids at positions 16 and 20 together form a ring
XXQGTFTSDYSKCLDEKRAKEFVQWLLDHHPSSGQPPPS

SEQ ID NO: 75 - protein, 40 aa, synthetic construct
  REGION 1..40: note = Trigonal agonist
  SITE 2: note = X is aminoisobutyric acid (Aib)
  SITE 16..20: note = amino acids at positions 16 and 20 together form a ring
YXQGTFTSDYSKYLDEKAAKEFVQWLLDHHPSSGQPPPSC

SEQ ID NO: 76 - protein, 40 aa, synthetic construct
  REGION 1..40: note = Trigonal agonist
  SITE 2: note = X is aminoisobutyric acid (Aib)
  SITE 16..20: note = amino acids at positions 16 and 20 together form a ring
YXQGTFTSDYSKYLDEKRAKDFVQWLLDHHPSSGQPPPSC

SEQ ID NO: 77 - protein, 40 aa, synthetic construct
  REGION 1..40: note = Trigonal agonist
  SITE 2: note = X is aminoisobutyric acid (Aib)
  SITE 16..20: note = amino acids at positions 16 and 20 together form a ring
YXQGTFTSDYSKYLDEKAAKDFVQWLLDHHPSSGQPPPSC

SEQ ID NO: 78 - protein, 31 aa, synthetic construct
  REGION 1..31: note = Trigonal agonist
  SITE 2: note = X is aminoisobutyric acid (Aib)
  SITE 16..20: note = amino acids at positions 16 and 20 together form a ring
HXQGTFTSDYSKYLDEKRQKEFVQWLLDTKC

SEQ ID NO: 79 - protein, 31 aa, synthetic construct
  REGION 1..31: note = Trigonal agonist
  SITE 2: note = X is aminoisobutyric acid (Aib)
  REGION 16..20: note = amino acids at positions 16 and 20 together form a ring
HXEGTFTSDYSIAMDEIHQKDFVNWLLAQKC

SEQ ID NO: 80 - protein, 31 aa, synthetic construct
  REGION 1..31: note = Trigonal agonist
  SITE 2: note = X is aminoisobutyric acid (Aib)
  SITE 16..20: note = amino acids at positions 16 and 20 together form a ring
HXEGTFTSDYSIAMDEIHQKDFVDWLLAEKC

SEQ ID NO: 81 - protein, 30 aa, synthetic construct
  REGION 1..30: note = Trigonal agonist
  SITE 1: note = X is 4-imidazoacetyl (CA)
  SITE 2: note = X is aminoisobutyric acid (Aib)
  SITE 16..20: note = amino acids at positions 16 and 20 together form a ring
XXQGTFTSDYSKYLDEKRQKEFVQWLLNTC

SEQ ID NO: 82 - protein, 30 aa, synthetic construct
  REGION 1..30: note = Trigonal agonist
  SITE 1: note = X is 4-imidazoacetyl (CA)
  SITE 2: note = X is aminoisobutyric acid (Aib)
  SITE 16..20: note = amino acids at positions 16 and 20 together form a ring
XXQGTFTSDYSKYLDEKRQKEFVQWLLDTC

SEQ ID NO: 83 - protein, 30 aa, synthetic construct
  REGION 1..30: note = Trigonal agonist
  SITE 1: note = X is 4-imidazoacetyl (CA)
  SITE 2: note = X is aminoisobutyric acid (Aib)
  SITE 16..20: note = amino acids at positions 16 and 20 together form a ring
XXEGTFTSDYSIAMDEIHQKDFVNWLLAQC

SEQ ID NO: 84 - protein, 30 aa, synthetic construct
  REGION 1..30: note = Trigonal agonist
  SITE 1: note = X is 4-imidazoacetyl (CA)
  SITE 2: note = X is aminoisobutyric acid (Aib)
  SITE 16..20: note = amino acids at positions 16 and 20 together form a ring
XXEGTFTSDYSIAMDEIHQKDFVDWLLAEC

SEQ ID NO: 85 - protein, 30 aa, synthetic construct
  REGION 1..30: note = Trigonal agonist
  SITE 1: note = X is 4-imidazoacetyl (CA)
  SITE 2: note = X is aminoisobutyric acid (Aib)
  SITE 16..20: note = amino acids at positions 16 and 20 together form a ring
XXQGTFTSDYSIAMDEIHQKDFVNWLLAQC

SEQ ID NO: 86 - protein, 30 aa, synthetic construct
  REGION 1..30: note = Trigonal agonist
  SITE 1: note = X is 4-imidazoacetyl (CA)
  SITE 2: note = X is aminoisobutyric acid (Aib)
  SITE 16..20: note = amino acids at positions 16 and 20 together form a ring
XXQGTFTSDYSKYLDEKRQKEFVNWLLAQC

SEQ ID NO: 87 - protein, 30 aa, synthetic construct
  REGION 1..30: note = Trigonal agonist
  SITE 1: note = X is 4-imidazoacetyl (CA)
  SITE 2: note = X is aminoisobutyric acid (Aib)
  SITE 16..20: note = amino acids at positions 16 and 20 together form a ring
XXQGTFTSDYSIAMDEIHQKDFVNWLLNTC

SEQ ID NO: 88 - protein, 31 aa, synthetic construct
  REGION 1..31: note = Trigonal agonist
  SITE 1: note = X is 4-imidazoacetyl (CA)
  SITE 2: note = X is aminoisobutyric acid (Aib)
  SITE 16..20: note = amino acids at positions 16 and 20 together form a ring
XXQGTFTSDYSKYLDEKRQKEFVQWLLNTKC

SEQ ID NO: 89 - protein, 31 aa, synthetic construct
  REGION 1..31: note = Trigonal agonist
  SITE 1: note = X is 4-imidazoacetyl (CA)
  SITE 2: note = X is aminoisobutyric acid (Aib)
  SITE 16..20: note = amino acids at positions 16 and 20 together form a ring
XXQGTFTSDYSKYLDEKRQKEFVQWLLDTKC

SEQ ID NO: 90 - protein, 31 aa, synthetic construct
  REGION 1..31: note = Trigonal agonist
  SITE 1: note = X is 4-imidazoacetyl (CA)
  SITE 2: note = X is aminoisobutyric acid (Aib)
  SITE 16..20: note = amino acids at positions 16 and 20 together form a ring
XXEGTFTSDYSIAMDEIHQKDFVNWLLAQKC

SEQ ID NO: 91 - protein, 31 aa, synthetic construct
  REGION 1..31: note = Trigonal agonist
  SITE 1: note = X is 4-imidazoacetyl (CA)
  SITE 2: note = X is aminoisobutyric acid (Aib)
  SITE 16..20: note = amino acids at positions 16 and 20 together form a ring
XXEGTFTSDYSIAMDEIHQKDFVDWLLAEKC

SEQ ID NO: 92 - protein, 31 aa, synthetic construct
  REGION 1..31: note = Trigonal agonist
  SITE 1: note = X is 4-imidazoacetyl (CA)
  SITE 2: note = X is aminoisobutyric acid (Aib)
  SITE 16..20: note = amino acids at positions 16 and 20 together form a ring
XXQGTFTSDYSIAMDEIHQKDFVNWLLAQKC

SEQ ID NO: 93 - protein, 31 aa, synthetic construct
  REGION 1..31: note = Trigonal agonist
  SITE 1: note = X is 4-imidazoacetyl (CA)
  SITE 2: note = X is aminoisobutyric acid (Aib)
  SITE 16..20: note = amino acids at positions 16 and 20 together form a ring
XXQGTFTSDYSKYLDEKRQKEFVNWLLAQKC

SEQ ID NO: 94 - protein, 31 aa, synthetic construct
  REGION 1..31: note = Trigonal agonist
  SITE 1: note = X is 4-imidazoacetyl (CA)
  SITE 2: note = X is aminoisobutyric acid (Aib)
  SITE 16..20: note = amino acids at positions 16 and 20 together form a ring
XXQGTFTSDYSIAMDEIHQKDFVNWLLNTKC

SEQ ID NO: 95 - protein, 39 aa, synthetic construct
  REGION 1..39: note = Trigonal agonist
  SITE 2: note = X is aminoisobutyric acid (Aib)
  SITE 16..20: note = amino acids at positions 16 and 20 together form a ring
YXQGTFTSDYSKYLDEKRAKEFVQWLLCHHPSSGQPPPS

SEQ ID NO: 96 - protein, 39 aa, synthetic construct
  REGION 1..39: note = Trigonal agonist
  SITE 2: note = X is aminoisobutyric acid (Aib)
  SITE 16..20: note = amino acids at positions 16 and 20 together form a ring
YXQGTFTSDYSKYLDEKRAKEFVQWLLDHCPSSGQPPPS

SEQ ID NO: 97 - protein, 39 aa, synthetic construct
  REGION 1..39: note = Trigonal agonist
  SITE 2: note = X is aminoisobutyric acid (Aib)
  SITE 16..20: note = amino acids at positions 16 and 20 together form a ring
YXQGTFTSDYSKYLDEKRAKEFVQWLLDCHPSSGQPPPS

SEQ ID NO: 98 - protein, 40 aa, synthetic construct
  REGION 1..40: note = Trigonal agonist
  SITE 2: note = X is aminoisobutyric acid (Aib)
  SITE 16..20: note = amino acids at positions 16 and 20 together form a ring
YXQGTFTSDYSKALDEKAAKEFVNWLLDHHPSSGQPPPSC

SEQ ID NO: 99 - protein, 40 aa, synthetic construct
  REGION 1..40: note = Trigonal agonist
  SITE 2: note = X is aminoisobutyric acid (Aib)
  SITE 16..20: note = amino acids at positions 16 and 20 together form a ring
YXQGTFTSDYSKALDEKAAKDFVNWLLDHHPSSGQPPPSC

SEQ ID NO: 100 - protein, 40 aa, synthetic construct
  REGION 1..40: note = Trigonal agonist
  SITE 2: note = X is aminoisobutyric acid (Aib)
  SITE 16..20: note = amino acids at positions 16 and 20 together form a ring
YXQGTFTSDYSKALDEKAAKEFVQWLLDQHPSSGQPPPSC

SEQ ID NO: 101 - protein, 40 aa, synthetic construct
  REGION 1..40: note = Trigonal agonist
  SITE 2: note = X is aminoisobutyric acid (Aib)
  REGION 16..20: note = amino acids at positions 16 and 20 together form a ring
YXQGTFTSDYSKALDEKAAKEFVNWLLDQHPSSGQPPPSC

SEQ ID NO: 102 - protein, 40 aa, synthetic construct
  REGION 1..40: note = Trigonal agonist
  SITE 2: note = X is aminoisobutyric acid (Aib)
  SITE 16..20: note = amino acids at positions 16 and 20 together form a ring
YXQGTFTSDYSKALDEKAAKDFVNWLLDQHPSSGQPPPSC

SEQ ID NO: 103 - protein, 30 aa, synthetic construct
  REGION 1..30: note = General Formula 1
  SITE 1: note = X is His (H), 4-imidazoacetyl (CA), or Tyr (Y)
  SITE 2: note = X is Gly (G), alpha-methyl-glutamic acid, or Aib (aminoisobutyric acid)
  SITE 3: note = X is Glu (E) or Gln (Q)
  SITE 7: note = X is Thr (T) or Ile (I)
  SITE 10: note = X is Leu (L), Tyr (Y), Lys (K), Cys (C), or Val (V)
  SITE 12: note = X is Lys (K), Ser (S), or Ile (I)
  SITE 13: note = X is Gln (Q), Tyr (Y), Ala (A), or Cys (C)
  SITE 14: note = X is Leu (L), Met (M), or Tyr (Y)
  SITE 15: note = X is Cys (C), Asp (D), Glu (E), or Leu (L)
  SITE 16: note = X is Gly (G), Glu (E), or Ser (S)
  SITE 17: note = X is Gln (Q), Arg (R), Ile (I), Glu (E), Cys (C), or Lys (K)
  SITE 18: note = X is Ala (A), Gln (Q), Arg (R), or His (H)
  SITE 19: note = X is Ala (A), Gln (Q), Cys (C), or Val (V)
  SITE 20: note = X is Lys (K), Gln (Q), or Arg (R)
  SITE 21: note = X is Glu (E), Gln (Q), Leu (L), Cys (C), or Asp (D)
  SITE 23: note = X is Ile (I) or Val (V)
  SITE 24: note = X is Ala (A), Gln (Q), Cys (C), Asn (N), Asp (D), or Glu (E)
  SITE 27: note = X is Val (V), Leu (L), Lys (K), or Met (M)
  SITE 28: note = X is Cys (C), Lys (K), Ala (A), Asn (N), or Asp (D)
  SITE 29: note = X is Cys (C), Gly (G), Gln (Q), Thr (T), Glu (E), or His (H)
  SITE 30: note = X is Cys (C), Gly (G), Lys (K), or His (H), or is absent; and X can be further linked to R1, wherein R1 is Cys (C), GKKNDWKHNIT, m-SSGAPPPS-n, or m-SSGQPPPS-n, or is absent, and wherein m is -Cys-, -Pro-, or -Gly-Pro-, and n is -Cys-, -Gly-, -Ser-, or -His
XXXGTFXSDXSXXXXXXXXXXFXXWLXXXX

SEQ ID NO: 104 - protein, 40 aa, synthetic construct
  REGION 1..40: note = General Formula 2
  SITE 1: note = X is His (H), 4-imidazoacetyl (CA), or Tyr (Y)
  SITE 2: note = X is Gly (G), alpha-methyl-glutamic acid, or Aib (aminoisobutyric acid)
  SITE 10: note = X is Tyr (Y) or Cys (C)
  SITE 13: note = X is Gln (Q), Tyr (Y), Ala (A), or Cys (C)
  SITE 14: note = X is Leu (L), Met (M), or Tyr (Y)
  SITE 15: note = X is Asp (D), Glu (E), or Leu (L)
  SITE 16: note = X is Gly (G), Glu (E), or Ser (S)
  SITE 17: note = X is Gln (Q), Arg (R), Ile (I), Glu (E), Cys (C), or Lys (K)
  SITE 18: note = X is Ala (A), Gln (Q), Arg (R), or His (H)
  SITE 19: note = X is Ala (A), Gln (Q), Cys (C), or Val (V)
  SITE 20: note = X is Lys (K), Gln (Q), or Arg (R)
  SITE 21: note = X is Glu (E), Gln (Q), Leu (L), Cys (C), or Asp (D)
  SITE 23: note = X is Ile (I) or Val (V)
  SITE 24: note = X is Ala (A), Gln (Q), Cys (C), Asn (N), or Glu (E)
  SITE 28: note = X is Cys (C), Lys (K), Asn (N), or Asp (D)
  SITE 29: note = X is Cys (C), Gly (G), Gln (Q), or His (H)
  SITE 30: note = X is Cys (C), Gly (G), Lys (K), or His (H)
  SITE 31: note = X is Pro (P) or Cys (C)
  SITE 40: note = X is Cys (C), or is absent
XXQGTFTSDXSKXXXXXXXXXFXXWLLXXXXSSGQPPPSX

SEQ ID NO: 105 - protein, 40 aa, synthetic construct
  REGION 1..40: note = General Formula 3
  SITE 1: note = X is His (H) or Tyr (Y)
  SITE 2: note = X is alpha-methyl-glutamic acid, or Aib (aminoisobutyric acid)
  SITE 13: note = X is Tyr (Y), Ala (A), or Cys (C)
  SITE 17: note = X is Arg (R), Cys (C), or Lys (K)
  SITE 18: note = X is Ala (A) or Arg (R)
  SITE 19: note = X is Ala (A) or Cys (C)
  SITE 21: note = X is Glu (E) or Asp (D)
  SITE 24: note = X is Gln (Q) or Asn (N)
  SITE 28: note = X is Cys (C) or Asp (D)
  SITE 29: note = X is Cys (C), Gln (Q), or His (H)
  SITE 30: note = X is Cys (C) or His (H)
  SITE 31: note = X is Pro (P) or Cys (C)
  SITE 40: note = X is Cys (C), or is absent
XXQGTFTSDYSKXLDEXXXKXFVXWLLXXXXSSGQPPPSX

SEQ ID NO: 106 - protein, 11 aa, synthetic construct
  REGION 1..11: note = R1
GKKNDWKHNIT

SEQ ID NO: 107 - protein, 8 aa, synthetic construct
  REGION 1..8: note = R1
SSGAPPPS

SEQ ID NO: 108 - protein, 8 aa, synthetic construct
  REGION 1..8: note = R1
SSGQPPPS

SEQ ID NO: 109 - protein, 9 aa, synthetic construct
  REGION 1..9: note = R1
CSSGQPPPS

SEQ ID NO: 110 - protein, 10 aa, synthetic construct
  REGION 1..10: note = R1
GPSSGAPPPS

SEQ ID NO: 111 - protein, 11 aa, synthetic construct
  REGION 1..11: note = R1
GPSSGAPPPSC

SEQ ID NO: 112 - protein, 9 aa, synthetic construct
  REGION 1..9: note = R1
PSSGAPPPS

SEQ ID NO: 113 - protein, 10 aa, synthetic construct
  REGION 1..10: note = R1
PSSGAPPPSG

SEQ ID NO: 114 - protein, 11 aa, synthetic construct
  REGION 1..11: note = R1
PSSGAPPPSHG

SEQ ID NO: 115 - protein, 10 aa, synthetic construct
  REGION 1..10: note = R1
PSSGAPPPSS

SEQ ID NO: 116 - protein, 9 aa, synthetic construct
  REGION 1..9: note = R1
PSSGQPPPS

SEQ ID NO: 117 - protein, 10 aa, synthetic construct
  REGION 1..10: note = R1
PSSGQPPPSC

SEQ ID NO: 118 - protein, 29 aa, Homo sapiens
HSQGTFTSDYSKYLDSRRAQDFVQWLMNT

SEQ ID NO: 119 - protein, 12 aa, Homo sapiens
ESKYGPPCPSCP

SEQ ID NO: 120 - protein, 11 aa, synthetic construct
  REGION 1..11: note = Variant of hinge region
ESKYGPPPSCP

SEQ ID NO: 121 - protein, 11 aa, synthetic construct
  REGION 1..11: note = Variant of hinge region
ESKYGPPCPSP

SEQ ID NO: 122 - protein, 10 aa, synthetic construct
  REGION 1..10: note = Variant of hinge region
ESKYGPPCPS

SEQ ID NO: 123 - protein, 10 aa, synthetic construct
  REGION 1..10: note = Variant of hinge region
ESKYGPPCPP

SEQ ID NO: 124 - protein, 8 aa, synthetic construct
  REGION 1..8: note = Variant of hinge region
KYGPPCPS

SEQ ID NO: 125 - protein, 8 aa, synthetic construct
  REGION 1..8: note = Variant of hinge region
ESKYGPPC

SEQ ID NO: 126 - protein, 7 aa, synthetic construct
  REGION 1..7: note = Variant of hinge region
EKYGPPC

SEQ ID NO: 127 - protein, 6 aa, synthetic construct
  REGION 1..6: note = Variant of hinge region
ESPSCP

SEQ ID NO: 128 - protein, 5 aa, synthetic construct
  REGION 1..5: note = Variant of hinge region
EPSCP

SEQ ID NO: 129 - protein, 4 aa, synthetic construct
  REGION 1..4: note = Variant of hinge region
PSCP

SEQ ID NO: 130 - protein, 10 aa, synthetic construct
  REGION 1..10: note = Variant of hinge region
ESKYGPPSCP

SEQ ID NO: 131 - protein, 9 aa, synthetic construct
  REGION 1..9: note = Variant of hinge region
KYGPPPSCP

SEQ ID NO: 132 - protein, 9 aa, synthetic construct
  REGION 1..9: note = Variant of hinge region
ESKYGPSCP

SEQ ID NO: 133 - protein, 8 aa, synthetic construct
  REGION 1..8: note = Variant of hinge region
ESKYGPPC

SEQ ID NO: 134 - protein, 7 aa, synthetic construct
  REGION 1..7: note = Variant of hinge region
KYGPPCP

SEQ ID NO: 135 - protein, 7 aa, synthetic construct
  REGION 1..7: note = Variant of hinge region
ESKPSCP

SEQ ID NO: 136 - protein, 6 aa, synthetic construct
  REGION 1..6: note = Variant of hinge region
ESPSCP

SEQ ID NO: 137 - protein, 4 aa, synthetic construct
  REGION 1..4: note = Variant of hinge region
EPSC

SEQ ID NO: 138 - skipped

SEQ ID NO: 139 - protein, 221 aa, Homo sapiens
PSCPAPEFLGGPSVFLFPPKPKDTLMISRTPEVTCVVVDVSQEDPEVQFNWYVDGVEVHNAKTKPREEQFNSTYRVVSVLTVLHQDWLNGKEYKCKVSNKGLPSSIEKTISKAKGQPREPQVYTLPPSQEEMTKNQVSLTCLVKGFYPSDIAVEWESNGQPENNYKTTPPVLDSDGSFFLYSRLTVDKSRWQEGNVFSCSVMHEALHNHYTQKSLSLSLGK

SEQ ID NO: 140 - protein, 442 aa, Homo sapiens
  REGION 1..442: note = Amino acids at position 1 to 442 form Human Immunoglobulin G4 Fc Fragment (homodimer)
  REGION 1..221: note = Amino acids at position 1 to 221 form one monomer
  REGION 222..442: note = Amino acids at position 222 to 442 form one monomer
  DISULFID 3..224: note = Amino acids at position 3 and position 224 form an inter-disulfide bond
  DISULFID 35..95: note = Amino acids at position 35 and position 95 form an intra-chain disulfide bond
  DISULFID 141..199: note = Amino acids at position 141 and position 199 form an intra-chain disulfide bond
  DISULFID 256..316: note = Amino acids at position 256 and position 316 form an intra-chain disulfide bond
  DISULFID 362..420: note = Amino acids at position 362 and position 420 form an intra-chain disulfide bond
PSCPAPEFLGGPSVFLFPPKPKDTLMISRTPEVTCVVVDVSQEDPEVQFNWYVDGVEVHNAKTKPREEQFNSTYRVVSVLTVLHQDWLNGKEYKCKVSNKGLPSSIEKTISKAKGQPREPQVYTLPPSQEEMTKNQVSLTCLVKGFYPSDIAVEWESNGQPENNYKTTPPVLDSDGSFFLYSRLTVDKSRWQEGNVFSCSVMHEALHNHYTQKSLSLSLGKPSCPAPEFLGGPSVFLFPPKPKDTLMISRTPEVTCVVVDVSQEDPEVQFNWYVDGVEVHNAKTKPREEQFNSTYRVVSVLTVLHQDWLNGKEYKCKVSNKGLPSSIEKTISKAKGQPREPQVYTLPPSQEEMTKNQVSLTCLVKGFYPSDIAVEWESNGQPENNYKTTPPVLDSDGSFFLYSRLTVDKSRWQEGNVFSCSVMHEALHNHYTQKSLSLSLGK